European Patent Specification EP 3 783 108 B1, published January 29, 2025. Title: METHOD FOR DETECTING TARGET NUCLEIC ACID AND NUCLEIC ACID PROBE USED THEREIN. Applicant: Eiken Kagaku Kabushiki Kaisha. Application not yet assigned. The sequence listing filed with the application follows.

SEQUENCE LISTING (50 sequences)

SEQ ID NO: 1 - DNA, 21 bp, Artificial Sequence
  Synthetic oligonucleotide
gcttttttttttttttttttc

SEQ ID NO: 2 - DNA, 20 bp, Artificial Sequence
  Synthetic oligonucleotide
aaaaaaaaaaaaaaaaaagc

SEQ ID NO: 3 - DNA, 21 bp, Artificial Sequence
  Synthetic oligonucleotide
  modified_base (20)..(20): I
gaaaaaaaaaaaaaaaaaanc

SEQ ID NO: 4 - DNA, 21 bp, Artificial Sequence
  Synthetic oligonucleotide
gaaaaaaaaaaaaaaaaaatc

SEQ ID NO: 5 - DNA, 21 bp, Artificial Sequence
  Synthetic oligonucleotide
gaaaaaaaaaaaaaaaaaacc

SEQ ID NO: 6 - DNA, 21 bp, Artificial Sequence
  Synthetic oligonucleotide
gaaaaaaaaaaaaaaaaaaac

SEQ ID NO: 7 - DNA, 21 bp, Artificial Sequence
  Synthetic oligonucleotide
  modified_base (20)..(20): Nebularine
gaaaaaaaaaaaaaaaaaanc

SEQ ID NO: 8 - DNA, 21 bp, Artificial Sequence
  Synthetic oligonucleotide
  modified_base (20)..(20): 2-dimethylaminomethyleneamino-6-methoxyaminopurine
gaaaaaaaaaaaaaaaaaanc

SEQ ID NO: 9 - DNA, 21 bp, Artificial Sequence
  Synthetic oligonucleotide
  modified_base (20)..(20): 3-Nitropyrrole
gaaaaaaaaaaaaaaaaaanc

SEQ ID NO: 10 - DNA, 21 bp, Artificial Sequence
  Synthetic oligonucleotide
gttcttttttttttttttttc

SEQ ID NO: 11 - DNA, 21 bp, Artificial Sequence
  Synthetic oligonucleotide
gttttcttttttttttttttc

SEQ ID NO: 12 - DNA, 21 bp, Artificial Sequence
  Synthetic oligonucleotide
gttttttcttttttttttttc

SEQ ID NO: 13 - DNA, 20 bp, Artificial Sequence
  Synthetic oligonucleotide
aaaaaaaaaaaaaaaagaac

SEQ ID NO: 14 - DNA, 20 bp, Artificial Sequence
  Synthetic oligonucleotide
aaaaaaaaaaaaaagaaaac

SEQ ID NO: 15 - DNA, 20 bp, Artificial Sequence
  Synthetic oligonucleotide
aaaaaaaaaaaagaaaaaac

SEQ ID NO: 16 - DNA, 21 bp, Artificial Sequence
  Synthetic oligonucleotide
  modified_base (18)..(18): I
gaaaaaaaaaaaaaaaanaac

SEQ ID NO: 17 - DNA, 21 bp, Artificial Sequence
  Synthetic oligonucleotide
  modified_base (16)..(16): I
gaaaaaaaaaaaaaanaaaac

SEQ ID NO: 18 - DNA, 21 bp, Artificial Sequence
  Synthetic oligonucleotide
  modified_base (14)..(14): I
gaaaaaaaaaaaanaaaaaac

SEQ ID NO: 19 - DNA, 22 bp, Artificial Sequence
  Synthetic oligonucleotide
gcctttttttttttttttttcc

SEQ ID NO: 20 - DNA, 20 bp, Artificial Sequence
  Synthetic oligonucleotide
aaaaaaaaaaaaaaaaaggc

SEQ ID NO: 21 - DNA, 21 bp, Artificial Sequence
  Synthetic oligonucleotide
  modified_base (20)..(20): I
gaaaaaaaaaaaaaaaaagnc

SEQ ID NO: 22 - DNA, 22 bp, Artificial Sequence
  Synthetic oligonucleotide
  modified_base (20)..(21): I
ggaaaaaaaaaaaaaaaaannc

SEQ ID NO: 23 - DNA, 425 bp, Mycoplasma pneumoniae
aattcgaatttgaaggcccaaggcctcacccaacccgcctacctcatcgccggtcttgacgttgtggccgaccacctcgtctttgcggcctttaaagcgggcgcggtggggtatgatatgacgactgattcgagcgcttcgacctacaaccaagcactcgcctggtcgaccacggccgggttggacagtgatggggggtacaaggccttggtggaaaacacggccgggctcaacggcccgattaatggcttgtttaccctgctcgacacctttgcgtatgtgacccccgtgagtgggatgaaaggggggagtcagaataatgaagaagtgcaaacgacttacccggtcaagtccgaccaaaaggccaccgccaaaattgcctccttaattaatgccagcccactcaacagttatggggatgatgg

SEQ ID NO: 24 - DNA, 21 bp, Artificial Sequence
  Synthetic oligonucleotide
tccgaccaaaaggccaccgcc

SEQ ID NO: 25 - DNA, 22 bp, Artificial Sequence
  Synthetic oligonucleotide
  modified_base (20)..(20): I
gtccgaccaaaaggccaccncc

SEQ ID NO: 26 - DNA, 664 bp, Mycobacterium tuberculosis
agttggcgcgcgacctgcatccggacgcgaacccgggcaacccggccgccggcgaacggttcaaggcggtttcggaggcgcataacgtgctgtcggatccggccaagcgcaaggagtacgacgaaacccgccgcctgttcgccggcggcgggttcggcggccgtcggttcgacagcggctttgggggcgggttcggcggtttcggggtcggtggagacggcgccgagttcaacctcaacgacttgttcgacgccgccagccgaaccggcggtaccaccatcggtgacttgttcggtggcttgttcggacgcggtggcagcgcccgtcccagccgcccgcgacgcggcaacgacctggagaccgagaccgagttggatttcgtggaggccgccaagggcgtggcgatgccgctgcgattaaccagcccggcgccgtgcaccaactgccatggcagcggggcccggccaggcaccagcccaaaggtgtgtcccacttgcaacgggtcgggcgtgatcaaccgcaatcagggcgcgttcggcttctccgagccgtgcaccgactgccgaggtagcggctcgatcatcgagcacccctgcgaggagtgcaaaggcaccggcgtgaccacccgcacccgaaccatcaacgtgcggatcccgcccggtgt

SEQ ID NO: 27 - DNA, 23 bp, Artificial Sequence
  Synthetic oligonucleotide
ccaagcgcaaggagtacgacgaa

SEQ ID NO: 28 - DNA, 27 bp, Artificial Sequence
  Synthetic oligonucleotide
gaacaagccaccgaacaagtcaccgat

SEQ ID NO: 29 - DNA, 15 bp, Artificial Sequence
  Synthetic oligonucleotide
cggtggagacggcgc

SEQ ID NO: 30 - DNA, 17 bp, Artificial Sequence
  Synthetic oligonucleotide
  modified_base (16)..(16): I
gtcggtggagacggcnc

SEQ ID NO: 31 - DNA, 18 bp, Artificial Sequence
  Synthetic oligonucleotide
  modified_base (15)..(15): I
  modified_base (17)..(17): I
ggtcggtggagacgncnc

SEQ ID NO: 32 - DNA, 21 bp, Artificial Sequence
  Synthetic oligonucleotide
gattttttttttttttttttc

SEQ ID NO: 33 - DNA, 21 bp, Artificial Sequence
  Synthetic oligonucleotide
ggttttttttttttttttttc

SEQ ID NO: 34 - DNA, 21 bp, Artificial Sequence
  Synthetic oligonucleotide
gtttttttttttttttttttc

SEQ ID NO: 35 - DNA, 21 bp, Artificial Sequence
  Synthetic oligonucleotide
gcttttttttttttttttttc

SEQ ID NO: 36 - DNA, 21 bp, Artificial Sequence
  Synthetic oligonucleotide
gaaaaaaaaaaaaaaaaaagc

SEQ ID NO: 37 - DNA, 21 bp, Artificial Sequence
  Synthetic oligonucleotide
  modified_base (20)..(20): I
gaaaaaaaaaaaaaaaaaanc

SEQ ID NO: 38 - DNA, 21 bp, Artificial Sequence
  Synthetic oligonucleotide
gaaaaaaaaaaaaaaaaaaac

SEQ ID NO: 39 - DNA, 21 bp, Artificial Sequence
  Synthetic oligonucleotide
gaaaaaaaaaaaaaaaaaatc

SEQ ID NO: 40 - DNA, 21 bp, Artificial Sequence
  Synthetic oligonucleotide
gaaaaaaaaaaaaaaaaaacc

SEQ ID NO: 41 - DNA, 21 bp, Artificial Sequence
  Synthetic oligonucleotide
gttattttttttttttttttc

SEQ ID NO: 42 - DNA, 21 bp, Artificial Sequence
  Synthetic oligonucleotide
gttgttttttttttttttttc

SEQ ID NO: 43 - DNA, 21 bp, Artificial Sequence
  Synthetic oligonucleotide
gtttttttttttttttttttc

SEQ ID NO: 44 - DNA, 21 bp, Artificial Sequence
  Synthetic oligonucleotide
gttcttttttttttttttttc

SEQ ID NO: 45 - DNA, 21 bp, Artificial Sequence
  Synthetic oligonucleotide
  modified_base (18)..(18): I
gaaaaaaaaaaaaaaaanaac

SEQ ID NO: 46 - DNA, 21 bp, Artificial Sequence
  Synthetic oligonucleotide
gttttattttttttttttttc

SEQ ID NO: 47 - DNA, 21 bp, Artificial Sequence
  Synthetic oligonucleotide
gttttgttttttttttttttc

SEQ ID NO: 48 - DNA, 21 bp, Artificial Sequence
  Synthetic oligonucleotide
gtttttttttttttttttttc

SEQ ID NO: 49 - DNA, 21 bp, Artificial Sequence
  Synthetic oligonucleotide
gttttcttttttttttttttc

SEQ ID NO: 50 - DNA, 21 bp, Artificial Sequence
  Synthetic oligonucleotide
  modified_base (16)..(16): I
gaaaaaaaaaaaaaanaaaac